European Patent Specification EP 3 454 910 B1, published November 5, 2025. Title: Treatment of Complement-Mediated Disorders. Applicant: CAMBRIDGE ENTERPRISE LIMITED THE SYDNEY CHILDREN'S HOSPITALS NETWORK (RANDWICK AND WESTMEAD) (INCORPORATING THE ROYAL ALEXANDRA HOSPITAL FOR CHILDREN). The sequence listing filed with the application follows.

SEQUENCE LISTING (12 sequences)

SEQ ID NO: 1 - DNA, 1752 bp, Homo sapiens
atgaagcttcttcatgttttcctgttatttctgtgcttccacttaaggttttgcaaggtcacttatacatctcaagaggatctggtggagaaaaagtgcttagcaaaaaaatatactcacctctcctgcgataaagtcttctgccagccatggcagagatgcattgagggcacctgtgtttgtaaactaccgtatcagtgcccaaagaatggcactgcagtgtgtgcaactaacaggagaagcttcccaacatactgtcaacaaaagagtttggaatgtcttcatccagggacaaagtttttaaataacggaacatgcacagccgaaggaaagtttagtgtttccttgaagcatggaaatacagattcagagggaatagttgaagtaaaacttgtggaccaagataagacaatgttcatatgcaaaagcagctggagcatgagggaagccaacgtggcctgccttgaccttgggtttcaacaaggtgctgatactcaaagaaggtttaagttgtctgatctctctataaattccactgaatgtctacatgtgcattgccgaggattagagaccagtttggctgaatgtacttttactaagagaagaactatgggttaccaggatttcgctgatgtggtttgttatacacagaaagcagattctccaatggatgacttctttcagtgtgtgaatgggaaatacatttctcagatgaaagcctgtgatggtatcaatgattgtggagaccaaagtgatgaactgtgttgtaaagcatgccaaggcaaaggcttccattgcaaatcgggtgtttgcattccaagccagtatcaatgcaatggtgaggtggactgcattacaggggaagatgaagttggctgtgcaggctttgcatctgtggctcaagaagaaacagaaattttgactgctgacatggatgcagaaagaagacggataaaatcattattacctaaactatcttgtggagttaaaaacagaatgcacattcgaaggaaacgaattgtgggaggaaagcgagcacaactgggagacctcccatggcaggtggcaattaaggatgccagtggaatcacctgtgggggaatttatattggtggctgttggattctgactgctgcacattgtctcagagccagtaaaactcatcgttaccaaatatggacaacagtagtagactggatacaccccgaccttaaacgtatagtaattgaatacgtggatagaattattttccatgaaaactacaatgcaggcacttaccaaaatgacatcgctttgattgaaatgaaaaaagacggaaacaaaaaagattgtgagctgcctcgttccatccctgcctgtgtcccctggtctccttacctattccaacctaatgatacatgcatcgtttctggctggggacgagaaaaagataacgaaagagtcttttcacttcagtggggtgaagttaaactaataagcaactgctctaagttttacggaaatcgtttctatgaaaaagaaatggaatgtgcaggtacatatgatggttccatcgatgcctgtaaaggggactctggaggccccttagtctgtatggatgccaacaatgtgacttatgtctggggtgttgtgagttggggggaaaactgtggaaaaccagagttcccaggtgtttacaccaaagtggccaattattttgactggattagctaccatgtaggaaggccttttatttctcagtacaatgtataa

SEQ ID NO: 2 - protein, 583 aa, Homo sapiens
MKLLHVFLLFLCFHLRFCKVTYTSQEDLVEKKCLAKKYTHLSCDKVFCQPWQRCIEGTCVCKLPYQCPKNGTAVCATNRRSFPTYCQQKSLECLHPGTKFLNNGTCTAEGKFSVSLKHGNTDSEGIVEVKLVDQDKTMFICKSSWSMREANVACLDLGFQQGADTQRRFKLSDLSINSTECLHVHCRGLETSLAECTFTKRRTMGYQDFADVVCYTQKADSPMDDFFQCVNGKYISQMKACDGINDCGDQSDELCCKACQGKGFHCKSGVCIPSQYQCNGEVDCITGEDEVGCAGFASVAQEETEILTADMDAERRRIKSLLPKLSCGVKNRMHIRRKRIVGGKRAQLGDLPWQVAIKDASGITCGGIYIGGCWILTAAHCLRASKTHRYQIWTTVVDWIHPDLKRIVIEYVDRIIFHENYNAGTYQNDIALIEMKKDGNKKDCELPRSIPACVPWSPYLFQPNDTCIVSGWGREKDNERVFSLQWGEVKLISNCSKFYGNRFYEKEMECAGTYDGSIDACKGDSGGPLVCMDANNVTYVWGVVSWGENCGKPEFPGVYTKVANYFDWISYHVGRPFISQYNV

SEQ ID NO: 3 - DNA, 1698 bp, Homo sapiens
aaggtcacttatacatctcaagaggatctggtggagaaaaagtgcttagcaaaaaaatatactcacctctcctgcgataaagtcttctgccagccatggcagagatgcattgagggcacctgtgtttgtaaactaccgtatcagtgcccaaagaatggcactgcagtgtgtgcaactaacaggagaagcttcccaacatactgtcaacaaaagagtttggaatgtcttcatccagggacaaagtttttaaataacggaacatgcacagccgaaggaaagtttagtgtttccttgaagcatggaaatacagattcagagggaatagttgaagtaaaacttgtggaccaagataagacaatgttcatatgcaaaagcagctggagcatgagggaagccaacgtggcctgccttgaccttgggtttcaacaaggtgctgatactcaaagaaggtttaagttgtctgatctctctataaattccactgaatgtctacatgtgcattgccgaggattagagaccagtttggctgaatgtacttttactaagagaagaactatgggttaccaggatttcgctgatgtggtttgttatacacagaaagcagattctccaatggatgacttctttcagtgtgtgaatgggaaatacatttctcagatgaaagcctgtgatggtatcaatgattgtggagaccaaagtgatgaactgtgttgtaaagcatgccaaggcaaaggcttccattgcaaatcgggtgtttgcattccaagccagtatcaatgcaatggtgaggtggactgcattacaggggaagatgaagttggctgtgcaggctttgcatctgtggctcaagaagaaacagaaattttgactgctgacatggatgcagaaagaagacggataaaatcattattacctaaactatcttgtggagttaaaaacagaatgcacattcgaaggaaacgaattgtgggaggaaagcgagcacaactgggagacctcccatggcaggtggcaattaaggatgccagtggaatcacctgtgggggaatttatattggtggctgttggattctgactgctgcacattgtctcagagccagtaaaactcatcgttaccaaatatggacaacagtagtagactggatacaccccgaccttaaacgtatagtaattgaatacgtggatagaattattttccatgaaaactacaatgcaggcacttaccaaaatgacatcgctttgattgaaatgaaaaaagacggaaacaaaaaagattgtgagctgcctcgttccatccctgcctgtgtcccctggtctccttacctattccaacctaatgatacatgcatcgtttctggctggggacgagaaaaagataacgaaagagtcttttcacttcagtggggtgaagttaaactaataagcaactgctctaagttttacggaaatcgtttctatgaaaaagaaatggaatgtgcaggtacatatgatggttccatcgatgcctgtaaaggggactctggaggccccttagtctgtatggatgccaacaatgtgacttatgtctggggtgttgtgagttggggggaaaactgtggaaaaccagagttcccaggtgtttacaccaaagtggccaattattttgactggattagctaccatgtaggaaggccttttatttctcagtacaatgtataa

SEQ ID NO: 4 - protein, 565 aa, Homo sapiens
KVTYTSQEDLVEKKCLAKKYTHLSCDKVFCQPWQRCIEGTCVCKLPYQCPKNGTAVCATNRRSFPTYCQQKSLECLHPGTKFLNNGTCTAEGKFSVSLKHGNTDSEGIVEVKLVDQDKTMFICKSSWSMREANVACLDLGFQQGADTQRRFKLSDLSINSTECLHVHCRGLETSLAECTFTKRRTMGYQDFADVVCYTQKADSPMDDFFQCVNGKYISQMKACDGINDCGDQSDELCCKACQGKGFHCKSGVCIPSQYQCNGEVDCITGEDEVGCAGFASVAQEETEILTADMDAERRRIKSLLPKLSCGVKNRMHIRRKRIVGGKRAQLGDLPWQVAIKDASGITCGGIYIGGCWILTAAHCLRASKTHRYQIWTTVVDWIHPDLKRIVIEYVDRIIFHENYNAGTYQNDIALIEMKKDGNKKDCELPRSIPACVPWSPYLFQPNDTCIVSGWGREKDNERVFSLQWGEVKLISNCSKFYGNRFYEKEMECAGTYDGSIDACKGDSGGPLVCMDANNVTYVWGVVSWGENCGKPEFPGVYTKVANYFDWISYHVGRPFISQYNV

SEQ ID NO: 5 - DNA, 27 bp, Artificial
  Primer sequence: FI-AAV-F
tctagaggatccgccaccatgaagctc

SEQ ID NO: 6 - DNA, 47 bp, Artificial
  Primer sequence: FI-AAV-R
aagcttggcggccgctcagacattgtgttgagaaacaagagaccttc

SEQ ID NO: 7 - DNA, 1752 bp, Homo sapiens
atgaagctgctgcatgtctttctgctgtttctgtgcttccatctgcggttctgtaaagtgacctatactagccaggaggatctggtggagaagaagtgtctggccaagaagtacacacacctgagctgcgacaaggtgttctgtcagccttggcagcggtgcatcgagggcacctgcgtgtgcaagctgccttaccagtgcccaaagaacggcaccgccgtgtgcgccacaaatcggagatcttttccaacatattgccagcagaagagcctggagtgtctgcaccccggcaccaagttcctgaacaatggcacctgcacagccgagggcaagttttctgtgagcctgaagcacggcaacacagatagcgagggcatcgtggaggtgaagctggtggaccaggataagaccatgttcatctgtaagagctcctggtccatgagggaggcaaacgtggcatgcctggatctgggattccagcagggagcagacacacagaggcgctttaagctgtccgacctgtctatcaatagcaccgagtgcctgcacgtgcactgtaggggcctggagacatccctggcagagtgcaccttcacaaagcggagaaccatgggctaccaggactttgccgacgtggtgtgctatacccagaaggccgatagccccatggacgatttctttcagtgcgtgaacggcaagtatatctcccagatgaaggcctgcgacggcatcaatgactgtggcgatcagtctgacgagctgtgctgtaaggcctgtcagggcaagggcttccactgcaagagcggcgtgtgcatcccttcccagtaccagtgcaacggcgaggtggattgtatcacaggagaggacgaagtgggatgcgcaggatttgcatctgtggcacaggaggagacagagatcctgacagccgacatggatgccgagaggcgccggatcaagtctctgctgcctaagctgagctgtggcgtgaagaatcggatgcacatcagaaggaagcgcatcgtgggaggcaagagggcacagctgggcgatctgccatggcaggtggccatcaaggacgcctctggcatcacctgcggcggcatctacatcggaggatgttggatcctgaccgcagcacactgcctgagagcaagcaagacacacaggtatcagatctggaccacagtggtggattggatccacccagacctgaagagaatcgtgatcgagtacgtggataggatcatctttcacgagaactacaatgccggcacatatcagaacgacatcgccctgatcgagatgaagaaggatggcaataagaaggactgtgagctgcccagatccatccctgcatgcgtgccatggagcccctatctgttccagcccaacgatacctgcatcgtgtccggatggggaagggagaaggacaatgagcgggtgttttctctgcagtggggcgaggtgaagctgatctccaactgttctaagttctacggcaataggttttatgagaaggagatggagtgcgccggcacctacgatggcagcatcgacgcctgtaagggcgattccggaggaccactggtgtgcatggacgcaaacaatgtgacatacgtgtggggagtggtgtcctggggagagaactgcggcaagccagagttccccggcgtatataccaaggtggccaattattttgattggatttcctaccacgtcggcaggccctttatttcccagtataatgtctaa

SEQ ID NO: 8 - DNA, 251 bp, Artificial
  HLP liver-specific promoter sequence
tgtttgctgcttgcaatgtttgcccattttagggtggacacaggacgctgtggtttctgagccagggggcgactcagatcccagccagtggacttagcccctgtttgctcctccgataactggggtgaccttggttaatattcaccagcagcctcccccgttgcccctctggatccactgcttaaatacggacgaggacagggccctgtctcctcagcttcaggcaccaccactgacctgggacagtgaat

SEQ ID NO: 9 - DNA, 447 bp, Artificial
  LP1 liver-specific promoter sequence
ccctaaaatgggcaaacattgcaagcagcaaacagcaaacacacagccctccctgcctgctgaccttggagctggggcagaggtcagagacctctctgggcccatgccacctccaacatccactcgaccccttggaatttcggtggagaggagcagaggttgtcctggcgtggtttaggtagtgtgagaggggaatgactcctttcggtaagtgcagtggaagctgtacactgcccaggcaaagcgtccgggcagcgtaggcgggcgactcagatcccagccagtggacttagcccctgtttgctcctccgataactggggtgaccttggttaatattcaccagcagcctcccccgttgcccctctggatccactgcttaaatacggacgaggacagggccctgtctcctcagcttcaggcaccaccactgacctgggacagtgaat

SEQ ID NO: 10 - DNA, 354 bp, Artificial
  HLP2 liver-specific promoter sequence
ccctaaaatgggcaaacattgcaagcagcaaacagcaaacacacagccctccctgcctgctgaccttggagctggggcagaggtcagacacctctctgggcccatgccacctccaactggacacaggacgctgtggtttctgagccagggggcgactcagatcccagccagtggacttagcccctgtttgctcctccgataactggggtgaccttggttaatattcaccagcagcctcccccgttgcccctctggatccactgcttaaatacggacgaggacagggccctgtctcctcagcttcaggcaccaccactgacctgggacagtgaatgatccccctgatctgcggcc

SEQ ID NO: 11 - protein, 736 aa, Artificial
  MutC capsid protein sequence
MAADGYLPDWLEDNLSEGIREWWALKPGAPKPKANQQKQDDGRGLVLPGYKYLGPFNGLDKGEPVNAADAAALEHDKAYDQQLQAGDNPYLRYNHADAEFQERLQEDTSFGGNLGRAVFQAKKRVLEPLGLVEEGAKTAPGKKRPVDQSPQEPDSSSGVGKSGKQPARKRLNFGQTGDSESVPDPQPLGEPPAAPTSLGSNTMASGGGAPMADNNEGADGVGNSSGNWHCDSQWLGDRVITTSTRTWALPTYNNHLYKQISSQSGASNDNHYFGYSTPWGYFDFNRFHCHFSPRDWQRLINNNWGFRPKKLSFKLFNIQVKEVTQNDGTTTIANNLTSTVQVFTDSEYQLPYVLGSAHQGCLPPFPADVFMVPQYGYLTLNNGSQAVGRSSFYCLEYFPSQMLRTGNNFQFSYTFEDVPFHSSYAHSQSLDRLMNPLIDQYLYYLNRTQGTTSGTTNQSRLLFSQAGPQSMSLQARNWLPGPCYRQQRLSKTANDNNNSNFPWTAASKYHLNGRDSLVNPGPAMASHKDDEEKFFPMHGNLIFGKEGTTASNAELDNVMITDEEEIRTTNPVATEQYGTVANNLQSSNTAPTTRTVNDQGALPGMVWQDRDVYLQGPIWAKIPHTDGHFHPSPLMGGFGLKHPPPQIMIKNTPVPANPPTTFSPAKFASFITQYSTGQVSVEIEWELQKENSKRWNPEIQYTSNYNKSVNVDFTVDTNGVYSEPRPIGTRYLTRNL

SEQ ID NO: 12 - protein, 736 aa, Artificial
  LK03 capsid protein sequence
MAADGYLPDWLEDNLSEGIREWWALQPGAPKPKANQQHQDNARGLVLPGYKYLGPGNGLDKGEPVNAADAAALEHDKAYDQQLKAGDNPYLKYNHADAEFQERLKEDTSFGGNLGRAVFQAKKRLLEPLGLVEEAAKTAPGKKRPVDQSPQEPDSSSGVGKSGKQPARKRLNFGQTGDSESVPDPQPLGEPPAAPTSLGSNTMASGGGAPMADNNEGADGVGNSSGNWHCDSQWLGDRVITTSTRTWALPTYNNHLYKQISSQSGASNDNHYFGYSTPWGYFDFNRFHCHFSPRDWQRLINNNWGFRPKKLSFKLFNIQVKEVTQNDGTTTIANNLTSTVQVFTDSEYQLPYVLGSAHQGCLPPFPADVFMVPQYGYLTLNNGSQAVGRSSFYCLEYFPSQMLRTGNNFQFSYTFEDVPFHSSYAHSQSLDRLMNPLIDQYLYYLNRTQGTTSGTTNQSRLLFSQAGPQSMSLQARNWLPGPCYRQQRLSKTANDNNNSNFPWTAASKYHLNGRDSLVNPGPAMASHKDDEEKFFPMHGNLIFGKEGTTASNAELDNVMITDEEEIRTTNPVATEQYGTVANNLQSSNTAPTTRTVNDQGALPGMVWQDRDVYLQGPIWAKIPHTDGHFHPSPLMGGFGLKHPPPQIMIKNTPVPANPPTTFSPAKFASFITQYSTGQVSVEIEWELQKENSKRWNPEIQYTSNYNKSVNVDFTVDTNGVYSEPRPIGTRYLTRPL